European Patent Specification EP 3 273 966 B1, published May 3, 2023. Title: INHIBITORS OF CYCLIN-DEPENDENT KINASES. Applicant: DANA-FARBER CANCER INSTITUTE, INC. Application PCT/US2016/024345. The sequence listing filed with the application follows.

SEQUENCE LISTING (279 sequences)

SEQ ID NO: 1 - protein, 18 aa, Artificial Sequence
  Synthetic Polypeptide
LMTGDTYTAHAGAKFPIK

SEQ ID NO: 2 - protein, 22 aa, Artificial Sequence
  Synthetic Polypeptide
YSLTVAVKTLKEDTMEVEEFLK

SEQ ID NO: 3 - protein, 25 aa, Artificial Sequence
  Synthetic Polypeptide
TVSVAVKCLKPDVLSQPEAMDDFIR

SEQ ID NO: 4 - protein, 10 aa, Artificial Sequence
  Synthetic Polypeptide
GTFGKVILVK

SEQ ID NO: 5 - protein, 10 aa, Artificial Sequence
  Synthetic Polypeptide
GTFGKVILVR

SEQ ID NO: 6 - protein, 19 aa, Artificial Sequence
  Synthetic Polypeptide
IGHYILGDTLGVGTFGKVK

SEQ ID NO: 7 - protein, 18 aa, Artificial Sequence
  Synthetic Polypeptide
VGKHELTGHKVAVKILNR

SEQ ID NO: 8 - protein, 8 aa, Artificial Sequence
  Synthetic Polypeptide
VAVKILNR

SEQ ID NO: 9 - protein, 16 aa, Artificial Sequence
  Synthetic Polypeptide
DLKPENVLLDAHMNAK

SEQ ID NO: 10 - protein, 16 aa, Artificial Sequence
  Synthetic Polypeptide
DLKSNNIFLHEGLTVK

SEQ ID NO: 11 - protein, 9 aa, Artificial Sequence
  Synthetic Polypeptide
FYIMMCKPK

SEQ ID NO: 12 - protein, 10 aa, Artificial Sequence
  Synthetic Polypeptide
FILALKVLFK

SEQ ID NO: 13 - protein, 16 aa, Artificial Sequence
  Synthetic Polypeptide
DIKPENLLLGSAGELK

SEQ ID NO: 14 - protein, 10 aa, Artificial Sequence
  Synthetic Polypeptide
GKFGNVYLAR

SEQ ID NO: 15 - protein, 12 aa, Artificial Sequence
  Synthetic Polypeptide
SHFIVALKVLFK

SEQ ID NO: 16 - protein, 16 aa, Artificial Sequence
  Synthetic Polypeptide
DLKPANILLDEHGHVR

SEQ ID NO: 17 - protein, 16 aa, Artificial Sequence
  Synthetic Polypeptide
DLKSNNIFLHEDLTVK

SEQ ID NO: 18 - protein, 9 aa, Artificial Sequence
  Synthetic Polypeptide
LFAVKCIPK

SEQ ID NO: 19 - protein, 17 aa, Artificial Sequence
  Synthetic Polypeptide
DLKPENLLYYSQDEESK

SEQ ID NO: 20 - protein, 12 aa, Artificial Sequence
  Synthetic Polypeptide
DLKPENLLLASK

SEQ ID NO: 21 - protein, 16 aa, Artificial Sequence
  Synthetic Polypeptide
IPTGQEYAAKIINTKK

SEQ ID NO: 22 - protein, 14 aa, Artificial Sequence
  Synthetic Polypeptide
TSTQEYAAKIINTK

SEQ ID NO: 23 - protein, 24 aa, Artificial Sequence
  Synthetic Polypeptide
IVEHQVLMKTVCGTPGYCAPEILR

SEQ ID NO: 24 - protein, 12 aa, Artificial Sequence
  Synthetic Polypeptide
GTQKPYALKVLK

SEQ ID NO: 25 - protein, 19 aa, Artificial Sequence
  Synthetic Polypeptide
DLKPENLLYATPAPDAPLK

SEQ ID NO: 26 - protein, 18 aa, Artificial Sequence
  Synthetic Polypeptide
LAYNENDNTYYAMKVLSK

SEQ ID NO: 27 - protein, 16 aa, Artificial Sequence
  Synthetic Polypeptide
DIKPSNLLVGEDGHIK

SEQ ID NO: 28 - protein, 16 aa, Artificial Sequence
  Synthetic Polypeptide
DLKPANLLISASGQLK

SEQ ID NO: 29 - protein, 16 aa, Artificial Sequence
  Synthetic Polypeptide
DLKPQNLLIDDKGTIK

SEQ ID NO: 30 - protein, 12 aa, Artificial Sequence
  Synthetic Polypeptide
DLKPQNLLIDDK

SEQ ID NO: 31 - protein, 12 aa, Artificial Sequence
  Synthetic Polypeptide
DLKVSNLLMTDK

SEQ ID NO: 32 - protein, 16 aa, Artificial Sequence
  Synthetic Polypeptide
DLKPANILVMGEGPER

SEQ ID NO: 33 - protein, 10 aa, Artificial Sequence
  Synthetic Polypeptide
LTGEVVALKK

SEQ ID NO: 34 - protein, 16 aa, Artificial Sequence
  Synthetic Polypeptide
DLKPQNLLINTEGAIK

SEQ ID NO: 35 - protein, 12 aa, Artificial Sequence
  Synthetic Polypeptide
NRETHEIVALKR

SEQ ID NO: 36 - protein, 11 aa, Artificial Sequence
  Synthetic Polypeptide
DLKPQNLLINR

SEQ ID NO: 37 - protein, 16 aa, Artificial Sequence
  Synthetic Polypeptide
DLKPQNILVTSSGQIK

SEQ ID NO: 38 - protein, 12 aa, Artificial Sequence
  Synthetic Polypeptide
DKNTNQIVAIKK

SEQ ID NO: 39 - protein, 16 aa, Artificial Sequence
  Synthetic Polypeptide
DLKPNNLLLDENGVLK

SEQ ID NO: 40 - protein, 11 aa, Artificial Sequence
  Synthetic Polypeptide
DMKAANVLITR

SEQ ID NO: 41 - protein, 12 aa, Artificial Sequence
  Synthetic Polypeptide
DIKCSNILLNNR

SEQ ID NO: 42 - protein, 12 aa, Artificial Sequence
  Synthetic Polypeptide
DIKPENLLLDER

SEQ ID NO: 43 - protein, 10 aa, Artificial Sequence
  Synthetic Polypeptide
LSKGDGLEFK

SEQ ID NO: 44 - protein, 8 aa, Artificial Sequence
  Synthetic Polypeptide
VAIKIISK

SEQ ID NO: 45 - protein, 19 aa, Artificial Sequence
  Synthetic Polypeptide
DLKPENVLLSSQEEDCLIK

SEQ ID NO: 46 - protein, 13 aa, Artificial Sequence
  Synthetic Polypeptide
DIKPDNFLMGIGR

SEQ ID NO: 47 - protein, 14 aa, Artificial Sequence
  Synthetic Polypeptide
DVKPDNFLMGLGKK

SEQ ID NO: 48 - protein, 15 aa, Artificial Sequence
  Synthetic Polypeptide
DVKPENFLVGRPGTK

SEQ ID NO: 49 - protein, 18 aa, Artificial Sequence
  Synthetic Polypeptide
GGPNIITLADIVKDPVSR

SEQ ID NO: 50 - protein, 14 aa, Artificial Sequence
  Synthetic Polypeptide
DVKPHNVMIDHQQK

SEQ ID NO: 51 - protein, 25 aa, Artificial Sequence
  Synthetic Polypeptide
LTHTDLKPENILFVQSDYTEAYNPK

SEQ ID NO: 52 - protein, 23 aa, Artificial Sequence
  Synthetic Polypeptide
YEIVGNLGEGTFGKVVECLDHAR

SEQ ID NO: 53 - protein, 16 aa, Artificial Sequence
  Synthetic Polypeptide
DIKCSNILLNNSGQIK

SEQ ID NO: 54 - protein, 22 aa, Artificial Sequence
  Synthetic Polypeptide
VSDFGLTKEASSTQDTGKLPVK

SEQ ID NO: 55 - protein, 7 aa, Artificial Sequence
  Synthetic Polypeptide
VAVKCIK

SEQ ID NO: 56 - protein, 21 aa, Artificial Sequence
  Synthetic Polypeptide
IDPVPNTHPLLVFVNPKSGGK

SEQ ID NO: 57 - protein, 25 aa, Artificial Sequence
  Synthetic Polypeptide
ATFSFCVSPLLVFVNSKSGDNQGVK

SEQ ID NO: 58 - protein, 14 aa, Artificial Sequence
  Synthetic Polypeptide
KGGSWIQEINVAEK

SEQ ID NO: 59 - protein, 13 aa, Artificial Sequence
  Synthetic Polypeptide
EHPFLVKGGEDLR

SEQ ID NO: 60 - protein, 24 aa, Artificial Sequence
  Synthetic Polypeptide
DVVHLDLKPQNILLTSESPLGDIK

SEQ ID NO: 61 - protein, 12 aa, Artificial Sequence
  Synthetic Polypeptide
YIKYNSNSGFVR

SEQ ID NO: 62 - protein, 22 aa, Artificial Sequence
  Synthetic Polypeptide
FLEDDTSDPTYTSALGGKIPIR

SEQ ID NO: 63 - protein, 16 aa, Artificial Sequence
  Synthetic Polypeptide
DLKPSNLLINTTCDLK

SEQ ID NO: 64 - protein, 16 aa, Artificial Sequence
  Synthetic Polypeptide
DLKPSNLLLNTTCDLK

SEQ ID NO: 65 - protein, 16 aa, Artificial Sequence
  Synthetic Polypeptide
DLKPSNLLVNENCELK

SEQ ID NO: 66 - protein, 31 aa, Artificial Sequence
  Synthetic Polypeptide
CIGEGQFGDVHQGIYMSPENPALAVAIKTCK

SEQ ID NO: 67 - protein, 18 aa, Artificial Sequence
  Synthetic Polypeptide
QEDGGVYSSSGLKQIPIK

SEQ ID NO: 68 - protein, 17 aa, Artificial Sequence
  Synthetic Polypeptide
TSVAVKTCKEDLPQELK

SEQ ID NO: 69 - protein, 18 aa, Artificial Sequence
  Synthetic Polypeptide
LIKDDEYNPCQGSKFPIK

SEQ ID NO: 70 - protein, 18 aa, Artificial Sequence
  Synthetic Polypeptide
IQSIAPSLQVITSKQRPR

SEQ ID NO: 71 - protein, 24 aa, Artificial Sequence
  Synthetic Polypeptide
VAIKTLKPGTMSPESFLEEAQIMK

SEQ ID NO: 72 - protein, 19 aa, Artificial Sequence
  Synthetic Polypeptide
QGAKFPIKWTAPEAALYGR

SEQ ID NO: 73 - protein, 14 aa, Artificial Sequence
  Synthetic Polypeptide
DTVTSELAAVKIVK

SEQ ID NO: 74 - protein, 16 aa, Artificial Sequence
  Synthetic Polypeptide
DIKGANLLLTLQGDVK

SEQ ID NO: 75 - protein, 10 aa, Artificial Sequence
  Synthetic Polypeptide
LDGCCYAVKR

SEQ ID NO: 76 - protein, 16 aa, Artificial Sequence
  Synthetic Polypeptide
DLKPVNIFLDSDDHVK

SEQ ID NO: 77 - protein, 16 aa, Artificial Sequence
  Synthetic Polypeptide
DLKPENILLDDYGHIR

SEQ ID NO: 78 - protein, 16 aa, Artificial Sequence
  Synthetic Polypeptide
DLKPENILLDDHGHIR

SEQ ID NO: 79 - protein, 17 aa, Artificial Sequence
  Synthetic Polypeptide
DIKPQNLLVDPDTAVLK

SEQ ID NO: 80 - protein, 17 aa, Artificial Sequence
  Synthetic Polypeptide
DIKPQNLLLDPDTAVLK

SEQ ID NO: 81 - protein, 14 aa, Artificial Sequence
  Synthetic Polypeptide
DKVSGDLVALKMVK

SEQ ID NO: 82 - protein, 16 aa, Artificial Sequence
  Synthetic Polypeptide
DIKGANILINDAGEVR

SEQ ID NO: 83 - protein, 15 aa, Artificial Sequence
  Synthetic Polypeptide
DLKPENIVLQDVGGK

SEQ ID NO: 84 - protein, 16 aa, Artificial Sequence
  Synthetic Polypeptide
WHNQETGEQIAIKQCR

SEQ ID NO: 85 - protein, 15 aa, Artificial Sequence
  Synthetic Polypeptide
DLKPENIVLQQGEQR

SEQ ID NO: 86 - protein, 19 aa, Artificial Sequence
  Synthetic Polypeptide
SGELVAVKVFNTTSYLRPR

SEQ ID NO: 87 - protein, 9 aa, Artificial Sequence
  Synthetic Polypeptide
DIKPGNIMR

SEQ ID NO: 88 - protein, 12 aa, Artificial Sequence
  Synthetic Polypeptide
WQGNDIVVKVLK

SEQ ID NO: 89 - protein, 15 aa, Artificial Sequence
  Synthetic Polypeptide
ISMADVKFSFQCPGR

SEQ ID NO: 90 - protein, 27 aa, Artificial Sequence
  Synthetic Polypeptide
AIQFLHQDSPSLIHGDIKSSNVLLDER

SEQ ID NO: 91 - protein, 12 aa, Artificial Sequence
  Synthetic Polypeptide
GYVNNTTVAVKK

SEQ ID NO: 92 - protein, 16 aa, Artificial Sequence
  Synthetic Polypeptide
DIKSANILLDEAFTAK

SEQ ID NO: 93 - protein, 17 aa, Artificial Sequence
  Synthetic Polypeptide
DLKPHNILISMPNAHGK

SEQ ID NO: 94 - protein, 18 aa, Artificial Sequence
  Synthetic Polypeptide
FVLDDQYTSSTGTKFPVK

SEQ ID NO: 95 - protein, 7 aa, Artificial Sequence
  Synthetic Polypeptide
VAIKTIR

SEQ ID NO: 96 - protein, 38 aa, Artificial Sequence
  Synthetic Polypeptide
ESIFFNSHNVSKPESSSVLTELDKIEGVFERPSDEVIR

SEQ ID NO: 97 - protein, 28 aa, Artificial Sequence
  Synthetic Polypeptide
QLASALSYLEDKDLVHGNVCTKNLLLAR

SEQ ID NO: 98 - protein, 20 aa, Artificial Sequence
  Synthetic Polypeptide
IGDFGLTKAIETDKEYYTVK

SEQ ID NO: 99 - protein, 31 aa, Artificial Sequence
  Synthetic Polypeptide
YDPEGDNTGEQVAVKSLKPESGGNHIADLKK

SEQ ID NO: 100 - protein, 10 aa, Artificial Sequence
  Synthetic Polypeptide
DLKPSNIVVK

SEQ ID NO: 101 - protein, 31 aa, Artificial Sequence
  Synthetic Polypeptide
YQQLKPIGSGAQGIVCAAFDTVLGINVAVKK

SEQ ID NO: 102 - protein, 14 aa, Artificial Sequence
  Synthetic Polypeptide
NVHTGELAAVKIIK

SEQ ID NO: 103 - protein, 16 aa, Artificial Sequence
  Synthetic Polypeptide
DIKGANILLTDHGDVK

SEQ ID NO: 104 - protein, 14 aa, Artificial Sequence
  Synthetic Polypeptide
NVNTGELAAIKVIK

SEQ ID NO: 105 - protein, 9 aa, Artificial Sequence
  Synthetic Polypeptide
ALYATKTLR

SEQ ID NO: 106 - protein, 11 aa, Artificial Sequence
  Synthetic Polypeptide
DIKPDNILIDR

SEQ ID NO: 107 - protein, 16 aa, Artificial Sequence
  Synthetic Polypeptide
DIKPDNILIDLDGHIK

SEQ ID NO: 108 - protein, 23 aa, Artificial Sequence
  Synthetic Polypeptide
EGAKFPIKWTAPEAINYGTFTIK

SEQ ID NO: 109 - protein, 16 aa, Artificial Sequence
  Synthetic Polypeptide
DIKPGNLLLTTGGTLK

SEQ ID NO: 110 - protein, 16 aa, Artificial Sequence
  Synthetic Polypeptide
NKETGALAAAKVIETK

SEQ ID NO: 111 - protein, 16 aa, Artificial Sequence
  Synthetic Polypeptide
DLKAGNVLMTLEGDIR

SEQ ID NO: 112 - protein, 16 aa, Artificial Sequence
  Synthetic Polypeptide
IMHRDVKPSNILVNSR

SEQ ID NO: 113 - protein, 12 aa, Artificial Sequence
  Synthetic Polypeptide
DVKPSNILVNSR

SEQ ID NO: 114 - protein, 18 aa, Artificial Sequence
  Synthetic Polypeptide
HQIMHRDVKPSNILVNSR

SEQ ID NO: 115 - protein, 12 aa, Artificial Sequence
  Synthetic Polypeptide
HAQSGTIMAVKR

SEQ ID NO: 116 - protein, 11 aa, Artificial Sequence
  Synthetic Polypeptide
DVKPSNVLINK

SEQ ID NO: 117 - protein, 14 aa, Artificial Sequence
  Synthetic Polypeptide
MVHKPSGQIMAVKR

SEQ ID NO: 118 - protein, 11 aa, Artificial Sequence
  Synthetic Polypeptide
DIKPSNILLDR

SEQ ID NO: 119 - protein, 12 aa, Artificial Sequence
  Synthetic Polypeptide
DVKPSNMLVNTR

SEQ ID NO: 120 - protein, 12 aa, Artificial Sequence
  Synthetic Polypeptide
HVPSGQIMAVKR

SEQ ID NO: 121 - protein, 16 aa, Artificial Sequence
  Synthetic Polypeptide
DVKPSNVLINALGQVK

SEQ ID NO: 122 - protein, 12 aa, Artificial Sequence
  Synthetic Polypeptide
DVKPSNILLDER

SEQ ID NO: 123 - protein, 15 aa, Artificial Sequence
  Synthetic Polypeptide
DVKGANLLIDSTGQR

SEQ ID NO: 124 - protein, 9 aa, Artificial Sequence
  Synthetic Polypeptide
IAIKEIPER

SEQ ID NO: 125 - protein, 31 aa, Artificial Sequence
  Synthetic Polypeptide
ELAVKQVQFDPDSPETSKEVNALECEIQLLK

SEQ ID NO: 126 - protein, 9 aa, Artificial Sequence
  Synthetic Polypeptide
DIKGANILR

SEQ ID NO: 127 - protein, 31 aa, Artificial Sequence
  Synthetic Polypeptide
ELASKQVQFDPDSPETSKEVSALECEIQLLK

SEQ ID NO: 128 - protein, 16 aa, Artificial Sequence
  Synthetic Polypeptide
DIKGANIFLTSSGLIK

SEQ ID NO: 129 - protein, 17 aa, Artificial Sequence
  Synthetic Polypeptide
DIKGDNVLINTYSGVLK

SEQ ID NO: 130 - protein, 17 aa, Artificial Sequence
  Synthetic Polypeptide
QVLGLGVNGKVLECFHR

SEQ ID NO: 131 - protein, 11 aa, Artificial Sequence
  Synthetic Polypeptide
CALKLLYDSPK

SEQ ID NO: 132 - protein, 9 aa, Artificial Sequence
  Synthetic Polypeptide
EVAVKIIDK

SEQ ID NO: 133 - protein, 19 aa, Artificial Sequence
  Synthetic Polypeptide
EVAVKIIDKTQLNSSSLQK

SEQ ID NO: 134 - protein, 21 aa, Artificial Sequence
  Synthetic Polypeptide
FIVHRDLKAENLLLDADMNIK

SEQ ID NO: 135 - protein, 16 aa, Artificial Sequence
  Synthetic Polypeptide
DLKAENLLLDADMNIK

SEQ ID NO: 136 - protein, 19 aa, Artificial Sequence
  Synthetic Polypeptide
EVAIKIIDKTQLNPTSLQK

SEQ ID NO: 137 - protein, 9 aa, Artificial Sequence
  Synthetic Polypeptide
EVAIKIIDK

SEQ ID NO: 138 - protein, 19 aa, Artificial Sequence
  Synthetic Polypeptide
EVAIKIIDKTQLNPSSLQK

SEQ ID NO: 139 - protein, 16 aa, Artificial Sequence
  Synthetic Polypeptide
DLKAENLLLDAEANIK

SEQ ID NO: 140 - protein, 16 aa, Artificial Sequence
  Synthetic Polypeptide
DLKPDNLLITSLGHIK

SEQ ID NO: 141 - protein, 11 aa, Artificial Sequence
  Synthetic Polypeptide
GAFGKVYLGQK

SEQ ID NO: 142 - protein, 8 aa, Artificial Sequence
  Synthetic Polypeptide
LYAVKVVK

SEQ ID NO: 143 - protein, 12 aa, Artificial Sequence
  Synthetic Polypeptide
DLKSSNILILQK

SEQ ID NO: 144 - protein, 24 aa, Artificial Sequence
  Synthetic Polypeptide
DLKSINILILEAIENHNLADTVLK

SEQ ID NO: 145 - protein, 10 aa, Artificial Sequence
  Synthetic Polypeptide
GELVAVKAAR

SEQ ID NO: 146 - protein, 21 aa, Artificial Sequence
  Synthetic Polypeptide
DLKSNNILLLQPIESDDMEHK

SEQ ID NO: 147 - protein, 9 aa, Artificial Sequence
  Synthetic Polypeptide
APVAIKVFK

SEQ ID NO: 148 - protein, 25 aa, Artificial Sequence
  Synthetic Polypeptide
LGEGGFSYVDLVEGLHDGHFYALKR

SEQ ID NO: 149 - protein, 34 aa, Artificial Sequence
  Synthetic Polypeptide
DLKPTNILLGDEGQPVLMDLGSMNQACIHVEGSR

SEQ ID NO: 150 - protein, 24 aa, Artificial Sequence
  Synthetic Polypeptide
DIKLENILLDSNGHVVLTDFGLSK

SEQ ID NO: 151 - protein, 24 aa, Artificial Sequence
  Synthetic Polypeptide
DLKLENVLLDSEGHIVLTDFGLSK

SEQ ID NO: 152 - protein, 22 aa, Artificial Sequence
  Synthetic Polypeptide
ETGQIVAIKQVPVESDLQEIIK

SEQ ID NO: 153 - protein, 16 aa, Artificial Sequence
  Synthetic Polypeptide
DIKAGNILLNTEGHAK

SEQ ID NO: 154 - protein, 22 aa, Artificial Sequence
  Synthetic Polypeptide
ESGQVVAIKQVPVESDLQEIIK

SEQ ID NO: 155 - protein, 36 aa, Artificial Sequence
  Synthetic Polypeptide
VVAIKIIDLEEAEDEIEDIQQEITVLSQCDSPYVTK

SEQ ID NO: 156 - protein, 16 aa, Artificial Sequence
  Synthetic Polypeptide
DIKAANVLLSEHGEVK

SEQ ID NO: 157 - protein, 39 aa, Artificial Sequence
  Synthetic Polypeptide
TQQVVAIKIIDLEEAEDEIEDIQQEITVLSQCDSSYVTK

SEQ ID NO: 158 - protein, 16 aa, Artificial Sequence
  Synthetic Polypeptide
DIKAANVLLSEQGDVK

SEQ ID NO: 159 - protein, 12 aa, Artificial Sequence
  Synthetic Polypeptide
DTGHVYAMKILR

SEQ ID NO: 160 - protein, 12 aa, Artificial Sequence
  Synthetic Polypeptide
DIKPDNLLLDSK

SEQ ID NO: 161 - protein, 12 aa, Artificial Sequence
  Synthetic Polypeptide
DTGHIYAMKILR

SEQ ID NO: 162 - protein, 12 aa, Artificial Sequence
  Synthetic Polypeptide
DIKPDNLLLDAK

SEQ ID NO: 163 - protein, 11 aa, Artificial Sequence
  Synthetic Polypeptide
DIKSQNIFLTK

SEQ ID NO: 164 - protein, 11 aa, Artificial Sequence
  Synthetic Polypeptide
SKNIFLTQNGK

SEQ ID NO: 165 - protein, 11 aa, Artificial Sequence
  Synthetic Polypeptide
DLKTQNVFLTR

SEQ ID NO: 166 - protein, 16 aa, Artificial Sequence
  Synthetic Polypeptide
DIKPANVFITATGVVK

SEQ ID NO: 167 - protein, 14 aa, Artificial Sequence
  Synthetic Polypeptide
AACLLDGVPVALKK

SEQ ID NO: 168 - protein, 11 aa, Artificial Sequence
  Synthetic Polypeptide
DLKTQNILLDK

SEQ ID NO: 169 - protein, 17 aa, Artificial Sequence
  Synthetic Polypeptide
RTEDDSLVVWKEVDLTR

SEQ ID NO: 170 - protein, 11 aa, Artificial Sequence
  Synthetic Polypeptide
DIKTLNIFLTK

SEQ ID NO: 171 - protein, 16 aa, Artificial Sequence
  Synthetic Polypeptide
DIKPGNLLVNSNCVLK

SEQ ID NO: 172 - protein, 34 aa, Artificial Sequence
  Synthetic Polypeptide
DVKAGNILLGEDGSVQIADFGVSAFLATGGDITR

SEQ ID NO: 173 - protein, 16 aa, Artificial Sequence
  Synthetic Polypeptide
DLKPSNLAVNEDCELK

SEQ ID NO: 174 - protein, 13 aa, Artificial Sequence
  Synthetic Polypeptide
QELNKTIWEVPER

SEQ ID NO: 175 - protein, 13 aa, Artificial Sequence
  Synthetic Polypeptide
QELNKTVWEVPQR

SEQ ID NO: 176 - protein, 16 aa, Artificial Sequence
  Synthetic Polypeptide
DLKPGNLAVNEDCELK

SEQ ID NO: 177 - protein, 16 aa, Artificial Sequence
  Synthetic Polypeptide
DLKPENIMLNHQGHVK

SEQ ID NO: 178 - protein, 10 aa, Artificial Sequence
  Synthetic Polypeptide
GGYGKVFQVR

SEQ ID NO: 179 - protein, 16 aa, Artificial Sequence
  Synthetic Polypeptide
DLKPENIMLSSQGHIK

SEQ ID NO: 180 - protein, 30 aa, Artificial Sequence
  Synthetic Polypeptide
IGQGASGTVFTATDVALGQEVAIKQINLQK

SEQ ID NO: 181 - protein, 12 aa, Artificial Sequence
  Synthetic Polypeptide
VMDPTKILITGK

SEQ ID NO: 182 - protein, 14 aa, Artificial Sequence
  Synthetic Polypeptide
SKLTDNLVALKEIR

SEQ ID NO: 183 - protein, 12 aa, Artificial Sequence
  Synthetic Polypeptide
DLKPQNLLINER

SEQ ID NO: 184 - protein, 12 aa, Artificial Sequence
  Synthetic Polypeptide
DLKPQNLLINEK

SEQ ID NO: 185 - protein, 14 aa, Artificial Sequence
  Synthetic Polypeptide
SKLTENLVALKEIR

SEQ ID NO: 186 - protein, 9 aa, Artificial Sequence
  Synthetic Polypeptide
EYAIKILEK

SEQ ID NO: 187 - protein, 16 aa, Artificial Sequence
  Synthetic Polypeptide
DLKPSNIFFTMDDVVK

SEQ ID NO: 188 - protein, 17 aa, Artificial Sequence
  Synthetic Polypeptide
ATGHEFAVKIMEVTAER

SEQ ID NO: 189 - protein, 16 aa, Artificial Sequence
  Synthetic Polypeptide
SGTPMQSAAKAPYLAK

SEQ ID NO: 190 - protein, 14 aa, Artificial Sequence
  Synthetic Polypeptide
VPHTQAVVLNSKDK

SEQ ID NO: 191 - protein, 23 aa, Artificial Sequence
  Synthetic Polypeptide
LLSVIVKCGDDLRQELLAFQVLK

SEQ ID NO: 192 - protein, 20 aa, Artificial Sequence
  Synthetic Polypeptide
VIFKCGDDLRQDMLTLQMIR

SEQ ID NO: 193 - protein, 32 aa, Artificial Sequence
  Synthetic Polypeptide
TEDGGKYPVIFKHGDDLRQDQLILQIISLMDK

SEQ ID NO: 194 - protein, 18 aa, Artificial Sequence
  Synthetic Polypeptide
TEDGGKYPVIFKHGDDLR

SEQ ID NO: 195 - protein, 42 aa, Artificial Sequence
  Synthetic Polypeptide
RPLWLNWENPDIMSELLFQNNEIIFKNGDDLRQDMLTLQIIR

SEQ ID NO: 196 - protein, 28 aa, Artificial Sequence
  Synthetic Polypeptide
VFGEDSVGVIFKNGDDLRQDMLTLQMLR

SEQ ID NO: 197 - protein, 16 aa, Artificial Sequence
  Synthetic Polypeptide
TKVNWLAHNVSKDNRQ

SEQ ID NO: 198 - protein, 14 aa, Artificial Sequence
  Synthetic Polypeptide
VNWLAHNVSKDNRQ

SEQ ID NO: 199 - protein, 9 aa, Artificial Sequence
  Synthetic Polypeptide
KKPLWLEFK

SEQ ID NO: 200 - protein, 18 aa, Artificial Sequence
  Synthetic Polypeptide
AKELPTLKDNDFINEGQK

SEQ ID NO: 201 - protein, 18 aa, Artificial Sequence
  Synthetic Polypeptide
AKDLPTFKDNDFLNEGQK

SEQ ID NO: 202 - protein, 15 aa, Artificial Sequence
  Synthetic Polypeptide
VKELPTLKDMDFLNK

SEQ ID NO: 203 - protein, 28 aa, Artificial Sequence
  Synthetic Polypeptide
TLVIKEVSSEDIADMHSNLSNYHQYIVK

SEQ ID NO: 204 - protein, 19 aa, Artificial Sequence
  Synthetic Polypeptide
GGKSGAAFYATEDDRFILK

SEQ ID NO: 205 - protein, 16 aa, Artificial Sequence
  Synthetic Polypeptide
DLKTSNLLLSHAGILK

SEQ ID NO: 206 - protein, 13 aa, Artificial Sequence
  Synthetic Polypeptide
KGTEELYAIKILK

SEQ ID NO: 207 - protein, 16 aa, Artificial Sequence
  Synthetic Polypeptide
DLKLDNVMLDSEGHIK

SEQ ID NO: 208 - protein, 14 aa, Artificial Sequence
  Synthetic Polypeptide
VKETGDLYAVKVLK

SEQ ID NO: 209 - protein, 8 aa, Artificial Sequence
  Synthetic Polypeptide
IYAMKVVK

SEQ ID NO: 210 - protein, 16 aa, Artificial Sequence
  Synthetic Polypeptide
DLKLDNVLLDSEGHIK

SEQ ID NO: 211 - protein, 24 aa, Artificial Sequence
  Synthetic Polypeptide
NIVHCDLKPENVLLASADPFPQVK

SEQ ID NO: 212 - protein, 9 aa, Artificial Sequence
  Synthetic Polypeptide
DVAVKVIDK

SEQ ID NO: 213 - protein, 9 aa, Artificial Sequence
  Synthetic Polypeptide
DVAIKVIDK

SEQ ID NO: 214 - protein, 24 aa, Artificial Sequence
  Synthetic Polypeptide
NIVHCDLKPENVLLASAEPFPQVK

SEQ ID NO: 215 - protein, 19 aa, Artificial Sequence
  Synthetic Polypeptide
VLLSEFRPSGELFAIKALK

SEQ ID NO: 216 - protein, 16 aa, Artificial Sequence
  Synthetic Polypeptide
DLKLDNLLLDTEGYVK

SEQ ID NO: 217 - protein, 16 aa, Artificial Sequence
  Synthetic Polypeptide
DLKLDNLLLDTEGFVK

SEQ ID NO: 218 - protein, 16 aa, Artificial Sequence
  Synthetic Polypeptide
IGDFGLVTSLKNDGKR

SEQ ID NO: 219 - protein, 13 aa, Artificial Sequence
  Synthetic Polypeptide
DLKPSNIFLVDTK

SEQ ID NO: 220 - protein, 20 aa, Artificial Sequence
  Synthetic Polypeptide
CFEISDADTKEVFAGKIVPK

SEQ ID NO: 221 - protein, 16 aa, Artificial Sequence
  Synthetic Polypeptide
DLKLGNLFLNEDLEVK

SEQ ID NO: 222 - protein, 19 aa, Artificial Sequence
  Synthetic Polypeptide
CNILHADIKPDNILVNESK

SEQ ID NO: 223 - protein, 15 aa, Artificial Sequence
  Synthetic Polypeptide
AAGIGKDFKENPNLR

SEQ ID NO: 224 - protein, 15 aa, Artificial Sequence
  Synthetic Polypeptide
FLSGLELVKQGAEAR

SEQ ID NO: 225 - protein, 14 aa, Artificial Sequence
  Synthetic Polypeptide
YIEDEDYYKASVTR

SEQ ID NO: 226 - protein, 18 aa, Artificial Sequence
  Synthetic Polypeptide
VAIKIIDKTQLDEENLKK

SEQ ID NO: 227 - protein, 16 aa, Artificial Sequence
  Synthetic Polypeptide
DMKSNNIFLHEGLTVK

SEQ ID NO: 228 - protein, 11 aa, Artificial Sequence
  Synthetic Polypeptide
DVKPDNMLLDK

SEQ ID NO: 229 - protein, 16 aa, Artificial Sequence
  Synthetic Polypeptide
LTDFGLSKEAIDHEKK

SEQ ID NO: 230 - protein, 17 aa, Artificial Sequence
  Synthetic Polypeptide
KVTRPDSGHLYAMKVLK

SEQ ID NO: 231 - protein, 16 aa, Artificial Sequence
  Synthetic Polypeptide
DLKPENILLDEEGHIK

SEQ ID NO: 232 - protein, 20 aa, Artificial Sequence
  Synthetic Polypeptide
DLKPSNILYVDESGNPECLR

SEQ ID NO: 233 - protein, 14 aa, Artificial Sequence
  Synthetic Polypeptide
VLGQGSFGKVFLVK

SEQ ID NO: 234 - protein, 16 aa, Artificial Sequence
  Synthetic Polypeptide
LTDFGLSKESIDHEKK

SEQ ID NO: 235 - protein, 20 aa, Artificial Sequence
  Synthetic Polypeptide
DLKPSNILYVDESGNPESIR

SEQ ID NO: 236 - protein, 15 aa, Artificial Sequence
  Synthetic Polypeptide
VLGVIDKVLLVMDTR

SEQ ID NO: 237 - protein, 9 aa, Artificial Sequence
  Synthetic Polypeptide
FYAVKVLQK

SEQ ID NO: 238 - protein, 28 aa, Artificial Sequence
  Synthetic Polypeptide
IVYRDLKPENILLDSVGHVVLTDFGLCK

SEQ ID NO: 239 - protein, 18 aa, Artificial Sequence
  Synthetic Polypeptide
AQNKETSVLAAAKVIDTK

SEQ ID NO: 240 - protein, 16 aa, Artificial Sequence
  Synthetic Polypeptide
DLKAGNILFTLDGDIK

SEQ ID NO: 241 - protein, 22 aa, Artificial Sequence
  Synthetic Polypeptide
DTVTIHSVGGTITILPTKTKPK

SEQ ID NO: 242 - protein, 17 aa, Artificial Sequence
  Synthetic Polypeptide
SYPYLFKGLEDLHLDER

SEQ ID NO: 243 - protein, 8 aa, Artificial Sequence
  Synthetic Polypeptide
VAVKVIDK

SEQ ID NO: 244 - protein, 12 aa, Artificial Sequence
  Synthetic Polypeptide
DLKPENVVFFEK

SEQ ID NO: 245 - protein, 21 aa, Artificial Sequence
  Synthetic Polypeptide
IIHTDIKPENILLSVNEQYIR

SEQ ID NO: 246 - protein, 8 aa, Artificial Sequence
  Synthetic Polypeptide
FVAMKVVK

SEQ ID NO: 247 - protein, 34 aa, Artificial Sequence
  Synthetic Polypeptide
DLKAGNILLGEDGSVQIADFGVSAFLATGGDVTR

SEQ ID NO: 248 - protein, 24 aa, Artificial Sequence
  Synthetic Polypeptide
YSVKVLPWLSPEVLQQNLQGYDAK

SEQ ID NO: 249 - protein, 14 aa, Artificial Sequence
  Synthetic Polypeptide
SVKASHILISVDGK

SEQ ID NO: 250 - protein, 22 aa, Artificial Sequence
  Synthetic Polypeptide
HTPTGTLVTIKITNLENCNEER

SEQ ID NO: 251 - protein, 28 aa, Artificial Sequence
  Synthetic Polypeptide
SIKASHILISGDGLVTLSGLSHLHSLVK

SEQ ID NO: 252 - protein, 17 aa, Artificial Sequence
  Synthetic Polypeptide
DLKPPNLLLVAGGTVLK

SEQ ID NO: 253 - protein, 16 aa, Artificial Sequence
  Synthetic Polypeptide
DIKAGNILLTEPGQVK

SEQ ID NO: 254 - protein, 16 aa, Artificial Sequence
  Synthetic Polypeptide
DVKAGNILLSEPGLVK

SEQ ID NO: 255 - protein, 24 aa, Artificial Sequence
  Synthetic Polypeptide
TGDLFAIKVFNNISFLRPVDVQMR

SEQ ID NO: 256 - protein, 11 aa, Artificial Sequence
  Synthetic Polypeptide
YAAVKIHQLNK

SEQ ID NO: 257 - protein, 31 aa, Artificial Sequence
  Synthetic Polypeptide
YLNEIKPPIIHYDLKPGNILLVDGTACGEIK

SEQ ID NO: 258 - protein, 11 aa, Artificial Sequence
  Synthetic Polypeptide
YVAVKIHQLNK

SEQ ID NO: 259 - protein, 31 aa, Artificial Sequence
  Synthetic Polypeptide
YLNEIKPPIIHYDLKPGNILLVNGTACGEIK

SEQ ID NO: 260 - protein, 18 aa, Artificial Sequence
  Synthetic Polypeptide
IGDFGLAKAVPEGHEYYR

SEQ ID NO: 261 - protein, 15 aa, Artificial Sequence
  Synthetic Polypeptide
DLKPQNILLSNPAGR

SEQ ID NO: 262 - protein, 10 aa, Artificial Sequence
  Synthetic Polypeptide
EVVAIKCVAK

SEQ ID NO: 263 - protein, 23 aa, Artificial Sequence
  Synthetic Polypeptide
NISHLDLKPQNILLSSLEKPHLK

SEQ ID NO: 264 - protein, 8 aa, Artificial Sequence
  Synthetic Polypeptide
GSFKTVYK

SEQ ID NO: 265 - protein, 17 aa, Artificial Sequence
  Synthetic Polypeptide
DLKCDNIFITGPTGSVK

SEQ ID NO: 266 - protein, 11 aa, Artificial Sequence
  Synthetic Polypeptide
IGDLGLATLKR

SEQ ID NO: 267 - protein, 37 aa, Artificial Sequence
  Synthetic Polypeptide
EVVAIKIIDLEEAEDEIEDIQQEITVLSQCDSPYITR

SEQ ID NO: 268 - protein, 12 aa, Artificial Sequence
  Synthetic Polypeptide
WISQDKEVAVKK

SEQ ID NO: 269 - protein, 20 aa, Artificial Sequence
  Synthetic Polypeptide
ISDFGLSKALGADDSYYTAR

SEQ ID NO: 270 - protein, 10 aa, Artificial Sequence
  Synthetic Polypeptide
QIDVAIKVLK

SEQ ID NO: 271 - protein, 29 aa, Artificial Sequence
  Synthetic Polypeptide
TGQLAAIKVMDVTEDEEEEIKLEINMLKK

SEQ ID NO: 272 - protein, 16 aa, Artificial Sequence
  Synthetic Polypeptide
DIKGQNVLLTENAEVK

SEQ ID NO: 273 - protein, 29 aa, Artificial Sequence
  Synthetic Polypeptide
TGQLAAIKVMDVTGDEEEEIKQEINMLKK

SEQ ID NO: 274 - protein, 346 aa, Homo sapiens
MALDVKSRAKRYEKLDFLGEGQFATVYKARDKNTNQIVAIKKIKLGHRSEAKDGINRTALREIKLLQELSHPNIIGLLDAFGHKSNISLVFDFMETDLEVIIKDNSLVLTPSHIKAYMLMTLQGLEYLHQHWILHRDLKPNNLLLDENGVLKLADFGLAKSFGSPNRAYTHQVVTRWYRAPELLFGARMYGVGVDMWAVGCILAELLLRVPFLPGDSDLDQLTRIFETLGTPTEEQWPDMCSLPDYVTFKSFPGIPLHHIFSAAGDDLLDLIQGLFLFNPCARITATQALKMKYFSNRPGPTPGCQLPRPNCPVETLKEQSNPALAIKRKRTEALEQGGLPKKLIF

SEQ ID NO: 275 - protein, 1490 aa, Homo sapiens
MPNSERHGGKKDGSGGASGTLQPSSGGGSSNSRERHRLVSKHKRHKSKHSKDMGLVTPEAASLGTVIKPLVEYDDISSDSDTFSDDMAFKLDRRENDERRGSDRSDRLHKHRHHQHRRSRDLLKAKQTEKEKSQEVSSKSGSMKDRISGSSKRSNEETDDYGKAQVAKSSSKESRSSKLHKEKTRKERELKSGHKDRSKSHRKRETPKSYKTVDSPKRRSRSPHRKWSDSSKQDDSPSGASYGQDYDLSPSRSHTSSNYDSYKKSPGSTSRRQSVSPPYKEPSAYQSSTRSPSPYSRRQRSVSPYSRRRSSSYERSGSYSGRSPSPYGRRRSSSPFLSKRSLSRSPLPSRKSMKSRSRSPAYSRHSSSHSKKKRSSSRSRHSSISPVRLPLNSSLGAELSRKKKERAAAAAAAKMDGKESKGSPVFLPRKENSSVEAKDSGLESKKLPRSVKLEKSAPDTELVNVTHLNTEVKNSSDTGKVKLDENSEKHLVKDLKAQGTRDSKPIALKEEIVTPKETETSEKETPPPLPTIASPPPPLPTTTPPPQTPPLPPLPPIPALPQQPPLPPSQPAFSQVPASSTSTLPPSTHSKTSAVSSQANSQPPVQVSVKTQVSVTAAIPHLKTSTLPPLPLPPLLPGDDDMDSPKETLPSKPVKKEKEQRTRHLLTDLPLPPELPGGDLSPPDSPEPKAITPPQQPYKKRPKICCPRYGERRQTESDWGKRCVDKFDIIGIIGEGTYGQVYKAKDKDTGELVALKKVRLDNEKEGFPITAIREIKILRQLIHRSVVNMKEIVTDKQDALDFKKDKGAFYLVFEYMDHDLMGLLESGLVHFSEDHIKSFMKQLMEGLEYCHKKNFLHRDIKCSNILLNNSGQIKLADFGLARLYNSEESRPYTNKVITLWYRPPELLLGEERYTPAIDVWSCGCILGELFTKKPIFQANLELAQLELISRLCGSPCPAVWPDVIKLPYFNTMKPKKQYRRRLREEFSFIPSAALDLLDHMLTLDPSKRCTAEQTLQSDFLKDVELSKMAPPDLPHWQDCHELWSKKRRRQRQSGVVVEEPPPSKTSRKETTSGTSTEPVKNSSPAPPQPAPGKVESGAGDAIGLADITQQLNQSELAVLLNLLQSQTDLSIPQMAQLLNIHSNPEMQQQLEALNQSISALTEATSQQQDSETMAPEESLKEAPSAPVILPSAEQTTLEASSTPADMQNILAVLLSQLMKTQEPAGSLEENNSDKNSGPQGPRRTPTMPQEEAAACPPHILPPEKRPPEPPGPPPPPPPPPLVEGDLSSAPQELNPAVTAALLQLLSQPEAEPPGHLPHEHQALRPMEYSTRPRPNRTYGNTDGPETGFSAIDTDERNSGPALTESLVQTLVKNRTFSGSLSHLGESSSYQGTGSVQFPGDQDLRFARVPLALHPVVGQPFLKAEGSSNSVVHAETKLQNYGELGPGTTGASSSGAGLHWGGPTQSSAYGKLYRGPTRVPPRGGRGRGVPY

SEQ ID NO: 276 - protein, 1512 aa, Homo sapiens
MPSSSDTALGGGGGLSWAEKKLEERRKRRRFLSPQQPPLLLPLLQPQLLQPPPPPPPLLFLAAPGTAAAAAAAAAASSSCFSPGPPLEVKRLARGKRRAGGRQKRRRGPRAGQEAEKRRVFSLPQPQQDGGGGASSGGGVTPLVEYEDVSSQSEQGLLLGGASAATAATAAGGTGGSGGSPASSSGTQRRGEGSERRPRRDRRSSSGRSKERHREHRRRDGQRGGSEASKSRSRHSHSGEERAEVAKSGSSSSSGGRRKSASATSSSSSSRKDRDSKAHRSRTKSSKEPPSAYKEPPKAYREDKTEPKAYRRRRSLSPLGGRDDSPVSHRASQSLRSRKSPSPAGGGSSPYSRRLPRSPSPYSRRRSPSYSRHSSYERGGDVSPSPYSSSSWRRSRSPYSPVLRRSGKSRSRSPYSSRHSRSRSRHRLSRSRSRHSSISPSTLTLKSSLAAELNKNKKARAAEAARAAEAAKAAEATKAAEAAAKAAKASNTSTPTKGNTETSASASQTNHVKDVKKIKIEHAPSPSSGGTLKNDKAKTKPPLQVTKVENNLIVDKATKKAVIVGKESKSAATKEESVSLKEKTKPLTPSIGAKEKEQHVALVTSTLPPLPLPPMLPEDKEADSLRGNISVKAVKKEVEKKLRCLLADLPLPPELPGGDDLSKSPEEKKTATQLHSKRRPKICGPRYGETKEKDIDWGKRCVDKFDIIGIIGEGTYGQVYKARDKDTGEMVALKKVRLDNEKEGFPITAIREIKILRQLTHQSIINMKEIVTDKEDALDFKKDKGAFYLVFEYMDHDLMGLLESGLVHFNENHIKSFMRQLMEGLDYCHKKNFLHRDIKCSNILLNNRGQIKLADFGLARLYSSEESRPYTNKVITLWYRPPELLLGEERYTPAIDVWSCGCILGELFTKKPIFQANQELAQLELISRICGSPCPAVWPDVIKLPYFNTMKPKKQYRRKLREEFVFIPAAALDLFDYMLALDPSKRCTAEQALQCEFLRDVEPSKMPPPDLPLWQDCHELWSKKRRRQKQMGMTDDVSTIKAPRKDLSLGLDDSRTNTPQGVLPSSQLKSQGSSNVAPVKTGPGQHLNHSELAILLNLLQSKTSVNMADFVQVLNIKVNSETQQQLNKINLPAGILATGEKQTDPSTPQQESSKPLGGIQPSSQTIQPKVETDAAQAAVQSAFAVLLTQLIKAQQSKQKDVLLEERENGSGHEASLQLRPPPEPSTPVSGQDDLIQHQDMRILELTPEPDRPRILPPDQRPPEPPEPPPVTEEDLDYRTENQHVPTTSSSLTDPHAGVKAALLQLLAQHQPQDDPKREGGIDYQAGDTYVSTSDYKDNFGSSSFSSAPYVSNDGLGSSSAPPLERRSFIGNSDIQSLDNYSTASSHSGGPPQPSAFSESFPSSVAGYGDIYLNAGPMLFSGDKDHRFEYSHGPIAVLANSSDPSTGPESTHPLPAKMHNYNYGGNLQENPSGPSLMHGQTWTSPAQGPGYSQGYRGHISTSTGRGRGRGLPY

SEQ ID NO: 277 - DNA, 20 bp, Artificial Sequence
  Synthetic Polynucleotide
ggcaggattgccatgagttg

SEQ ID NO: 278 - DNA, 20 bp, Artificial Sequence
  Synthetic Polynucleotide
ggcaagattgtcatgagtta

SEQ ID NO: 279 - protein, 4 aa, Artificial Sequence
  Synthetic Polypeptide
  misc_feature (1)..(1): Xaa can be phosphorylated serine or phosphorylated threonine
  misc_feature (3)..(3): Xaa can be any naturally occurring amino acid
  misc_feature (4)..(4): Xaa can be lysine or arginine
XPXX